European Patent Application EP 4 194 467 A1, published June 14, 2023. Title: ANTI-MESOTHELIN CHIMERIC ANTIBODY RECEPTOR SPECIFICALLY BINDING TO MESOTHELIN. Applicant: Cellengene Inc. The sequence listing filed with the application follows.

SEQUENCE LISTING (40 sequences)

SEQ ID NO: 1 - protein, 5 aa, Artificial Sequence
  MSLN34 HCDR1
DYGMH

SEQ ID NO: 2 - protein, 17 aa, Artificial Sequence
  MSLN34 HCDR2
SIYGSGGHTGYADSVKG

SEQ ID NO: 3 - protein, 12 aa, Artificial Sequence
  MSLN34 HCDR3
QHAYRYSYAFDV

SEQ ID NO: 4 - protein, 11 aa, Artificial Sequence
  MSLN34 LCDR1
RASQSISNWLN

SEQ ID NO: 5 - protein, 7 aa, Artificial Sequence
  MSLN34 LCDR2
ATSSLQS

SEQ ID NO: 6 - protein, 9 aa, Artificial Sequence
  MSLN34 LCDR3
QQSYSFPFT

SEQ ID NO: 7 - protein, 5 aa, Artificial Sequence
  MSLN37 HCDR1
SYAMH

SEQ ID NO: 8 - protein, 17 aa, Artificial Sequence
  MSLN37 HCDR2
GISGSGGTTYYADSVKG

SEQ ID NO: 9 - protein, 12 aa, Artificial Sequence
  MSLN37 HCDR3
EVEGQSQEYFDI

SEQ ID NO: 10 - protein, 11 aa, Artificial Sequence
  MSLN37 LCDR1
RASQSIANYLN

SEQ ID NO: 11 - protein, 7 aa, Artificial Sequence
  MSLN37 LCDR2
AASNLQS

SEQ ID NO: 12 - protein, 9 aa, Artificial Sequence
  MSLN37 LCDR3
QQSYSFPYT

SEQ ID NO: 13 - protein, 5 aa, Artificial Sequence
  MSLN38 HCDR1
SYAMS

SEQ ID NO: 14 - protein, 17 aa, Artificial Sequence
  MSLN38 HCDR2
GISGSGGSTGYADSVKG

SEQ ID NO: 15 - protein, 12 aa, Artificial Sequence
  MSLN38 HCDR3
HGQVGGISVFDI

SEQ ID NO: 16 - protein, 11 aa, Artificial Sequence
  MSLN38 LCDR1
RASQSISNWLN

SEQ ID NO: 17 - protein, 7 aa, Artificial Sequence
  MSLN38 LCDR2
ATSRLQS

SEQ ID NO: 18 - protein, 9 aa, Artificial Sequence
  MSLN38 LCDR3
QQSYSFPWT

SEQ ID NO: 19 - protein, 121 aa, Artificial Sequence
  MSLN34 VH
EVQLVESGGGLVQPGGSLRLSCAASGFTFSDYGMHWVRQAPGKGLEWVSSIYGSGGHTGYADSVKGRFTISRDNSKNTLYLQMNSLRAEDTAVYYCAKQHAYRYSYAFDVWGQGTLVTVSS

SEQ ID NO: 20 - protein, 107 aa, Artificial Sequence
  MSLN34 VL
DIQMTQSPSSLSASVGDRVTITCRASQSISNWLNWYQQKPGKAPKLLIYATSSLQSGVPSRFSGSGSGTDFTLTISSLQPEDFATYYCQQSYSFPFTFGQGTKVEIK

SEQ ID NO: 21 - protein, 121 aa, Artificial Sequence
  MSLN37 VH
EVQLVESGGGLVQPGGSLRLSCAASGFTFSSYAMHWVRQAPGKGLEWVSGISGSGGTTYYADSVKGRFTISRDNSKNTLYLQMNSLRAEDTAVYYCAKEVEGQSQEYFDIWGQGTLVTVSS

SEQ ID NO: 22 - protein, 107 aa, Artificial Sequence
  MSLN37 VL
DIQMTQSPSSLSASVGDRVTITCRASQSIANYLNWYQQKPGKAPKLLIYAASNLQSGVPSRFSGSGSGTDFTLTISSLQPEDFATYYCQQSYSFPYTFGQGTKVEIK

SEQ ID NO: 23 - protein, 121 aa, Artificial Sequence
  MSLN38 VH
EVQLVESGGGLVQPGGSLRLSCAASGFTFSSYAMSWVRQAPGKGLEWVSGISGSGGSTGYADSVKGRFTISRDNSKNTLYLQMNSLRAEDTAVYYCAKHGQVGGISVFDIWGQGTLVTVSS

SEQ ID NO: 24 - protein, 107 aa, Artificial Sequence
  MSLN38 VL
DIQMTQSPSSLSASVGDRVTITCRASQSISNWLNWYQQKPGKAPKLLIYATSRLQSGVPSRFSGSGSGTDFTLTISSLQPEDFATYYCQQSYSFPWTFGQGTKVEIK

SEQ ID NO: 25 - DNA, 63 bp, Artificial Sequence
  CD8
atggccttaccagtgaccgccttgctcctgccgctggccttgctgctccacgccgccaggccg

SEQ ID NO: 26 - DNA, 738 bp, Artificial Sequence
  MSLN34 scFv
gaagtacagttggtcgaaagtggcggtggcctcgtgcaaccgggtggttcactgcgtctgagctgcgccgcctcgggttttactttctctgattatggtatgcactgggttcgtcaggcgccgggcaagggtctcgaatgggtttcatctatctacggttctggtggtcacactggttatgccgattcagtgaagggtcgctttaccatttcccgtgacaactctaagaatactctgtatctgcagatgaactcgctgcgtgccgaagacacggccgtctattattgcgccaaacagcatgcataccgttactcttacgcattcgatgtttggggtcagggcactttagtgaccgtctcatcgggtggaggcggttcaggcggaggtggatccggcggtggcggatcggacattcaaatgacgcagagtccctcctcactgagtgctagcgtgggcgatcgtgtgacaattacttgtcgcgctagccagtctatctctaattggctgaactggtatcagcagaaaccgggcaaggcgccaaaattgctgatttacgcaacttcctctctgcagtctggtgtaccgtcccgtttctctggcagcggttctggtacggattttaccctgaccatctcaagcctccagcctgaagattttgccacctattattgtcagcaatcttactcttttccgtttacgttcgggcagggaactaaagtggaaattaaagccagcacc

SEQ ID NO: 27 - DNA, 738 bp, Artificial Sequence
  MSLN38 scFv
gaagtacagttggtcgaaagtggcggtggcctcgtgcaaccgggtggttcactgcgtctgagctgcgccgcctcgggttttactttctcttcttatgcaatgtcttgggttcgtcaggcgccgggcaagggtctcgaatgggtttcaggtatctctggttctggtggttctactggttatgccgattcagtgaagggtcgctttaccatttcccgtgacaactctaagaatactctgtatctgcagatgaactcgctgcgtgccgaagacacggccgtctattattgcgccaaacatggtcaggttggtggtatctctgttttcgatatctggggtcagggcactttagtgaccgtctcatcgggtggaggcggttcaggcggaggtggatccggcggtggcggatcggacattcaaatgacgcagagtccctcctcactgagtgctagcgtgggcgatcgtgtgacaattacttgtcgcgctagccagtctatctctaattggctgaactggtatcagcagaaaccgggcaaggcgccaaaattgctgatttacgcaacttcccgtctgcagtctggtgtaccgtcccgtttctctggcagcggttctggtacggattttaccctgaccatctcaagcctccagcctgaagattttgccacctattattgtcagcaatcttactcttttccgtggacgttcgggcagggaactaaagtggaaattaaagccagcacc

SEQ ID NO: 28 - DNA, 135 bp, Artificial Sequence
  CD8 hinge
accacgacgccagcgccgcgaccaccaacaccggcgcccaccatcgcgtcgcagcccctgtccctgcgcccagaggcgtgccggccagcggcggggggcgcagtgcacacgagggggctggacttcgcctgtgat

SEQ ID NO: 29 - DNA, 72 bp, Artificial Sequence
  CD8 TM(TransMembrane)
atctacatctgggcgcccttggccgggacttgtggggtccttctcctgtcactggttatcaccctttactgc

SEQ ID NO: 30 - DNA, 126 bp, Artificial Sequence
  4-1BB
aaacggggcagaaagaaactcctgtatatattcaaacaaccatttatgagaccagtacaaactactcaagaggaagatggctgtagctgccgatttccagaagaagaagaaggaggatgtgaactg

SEQ ID NO: 31 - DNA, 337 bp, Artificial Sequence
  CD3z
agagtgaagttcagcaggagcgcagacgcccccgcgtacacagcagggccagaaccagctctataacgagctcaatctaggacgaagagaggagtacgatgttttggacaagagacgtggccgggaccctgagatggggggaaagccgagaaggaagaaccctcaggaaggcctgtacaatgaactgcagaaagataagatggcggaggcctacagtgagattgggatgaaaggcgagcgccggaggggcaaggggcacgatggcctttaccagggtctcagtacagccaccaaggacacctacgacgcccttcacatgcaggccctgccccctcgc

SEQ ID NO: 32 - protein, 5 aa, Artificial Sequence
  MSLN3 HCDR1
DYAMS

SEQ ID NO: 33 - protein, 17 aa, Artificial Sequence
  MSLN3 HCDR2
AISSSGGTTYYADSVKG

SEQ ID NO: 34 - protein, 12 aa, Artificial Sequence
  MSLN3 HCDR3
EEEGEWREYFDV

SEQ ID NO: 35 - protein, 11 aa, Artificial Sequence
  MSLN3 LCDR1
RASQSISSYLN

SEQ ID NO: 36 - protein, 7 aa, Artificial Sequence
  MSLN3 LCDR2
ATSTLQS

SEQ ID NO: 37 - protein, 9 aa, Artificial Sequence
  MSLN3 LCDR3
QQSYTFPYT

SEQ ID NO: 38 - protein, 121 aa, Artificial Sequence
  MSLN3 VH
EVQLVESGGGLVQPGGSLRLSCAASGFTFSDYAMSWVRQAPGKGLEWVSAISSSGGTTYYADSVKGRFTISRDNSKNTLYLQMNSLRAEDTAVYYCAKEEEGEWREYFDVWGQGTLVTVSS

SEQ ID NO: 39 - protein, 107 aa, Artificial Sequence
  MSLN3 VL
DIQMTQSPSSLSASVGDRVTITCRASQSISSYLNWYQQKPGKAPKLLIYATSTLQSGVPSRFSGSGSGTDFTLTISSLQPEDFATYYCQQSYTFPYTFGQGTKVEIK

SEQ ID NO: 40 - protein, 630 aa, Artificial Sequence
  MSLN(mesothelin)
MALPTARPLLGSCGTPALGSLLFLLFSLGWVQPSRTLAGETGQEAAPLDGVLANPPNISSLSPRQLLGFPCAEVSGLSTERVRELAVALAQKNVKLSTEQLRCLAHRLSEPPEDLDALPLDLLLFLNPDAFSGPQACTRFFSRITKANVDLLPRGAPERQRLLPAALACWGVRGSLLSEADVRALGGLACDLPGRFVAESAEVLLPRLVSCPGPLDQDQQEAARAALQGGGPPYGPPSTWSVSTMDALRGLLPVLGQPIIRSIPQGIVAAWRQRSSRDPSWRQPERTILRPRFRREVEKTACPSGKKAREIDESLIFYKKWELEACVDAALLATQMDRVNAIPFTYEQLDVLKHKLDELYPQGYPESVIQHLGYLFLKMSPEDIRKWNVTSLETLKALLEVNKGHEMSPQAPRRPLPQVATLIDRFVKGRGQLDKDTLDTLTAFYPGYLCSLSPEELSSVPPSSIWAVRPQDLDTCDPRQLDVLYPKARLAFQNMNGSEYFVKIQSFLGGAPTEDLKALSQQNVSMDLATFMKLRTDAVLPLTVAEVQKLLGPHVEGLKAEERHRPVRDWILRQRQDDLDTLGLGLQGGIPNGYLVLDLSMQEALSGTPCLLGPGPVLTVLALLLASTLA